European Patent Application EP 4 293 129 A2, published December 20, 2023. Title: METHODS AND AGRICULTURAL COMPOSITIONS FOR PREVENTING OR CONTROLLING PLANT DISEASES. Applicant: Tenfold Technologies, LLC. The sequence listing filed with the application follows.

SEQUENCE LISTING (32 sequences)

SEQ ID NO: 1 - DNA, 1147 bp, Paenibacillus sp.
  source 1..1147: mol_type = genomic DNA
gagtttgatcctggctcaggacgaacgctggcggcgtgcctaatacatgcaagtcgagcggggttatgtagaagcttgcttctaaataacctagcggcggacgggtgagtaacacgtaggcaacctgcccacaagacagggataactaccggaaacggtagctaatacccgatacatccttttcctgcatgggagagggaggaaagacggagcaatctgtcacttgtggatgggcctgcggcgcattagctagttggtggggtaaaggcctaccaaggcgacgatgcgtagccgacctgagagggtgatcggccacactgggactgagacacggcccagactcctacgggaggcagcagtagggaatcttccgcaatgggcgaaagcctgacggagcaacgccgcgtgagtgatgaaggttttcggatcgtaaagctctgttgccagggaagaacgtcttgtagagtaactgctacaagagtgacggtacctgagaagaaagccccggctaactacgtgccagcagccgcggtaatacgtagggggcaagcgttgtccggaattattgggcgtaaagcgcgcgcaggcggctctttaagtctggtgtttaatcccgaggctcaacttcgggtcgcactggaaactggggagcttgagtgcagaagaggagagtggaattccacgtgtagcggtgaaatgcgtagagatgtggaggaacaccagtggcgaaggcgactctctgggctgtaactgacgctgaggcgcgaaagcgtggggagcaaacaggattagataccctggtagtccacgccgtaaacgatgaatgctaggtgttaggggtttcgatacccttggtgccgaagttaacacattaagcattccgcctggggagtacggtcgcaagactgaaactcaaaggaattgacggggacccgcacaagcagtggagtatgtggtttaattcgaagcaacgcgaagaaccttaccaggtcttgacatccctctgaccgctgtagagatatggctttccttcgggacagaggagacaggtggtgcatggttgtcgtcagctcgtgtcgtgagatgttgggttaagtcccgcaacgagcgcaacccttatgcttagttgccagcaggtcaagctggg

SEQ ID NO: 2 - DNA, 1025 bp, Bacillus sp.
  source 1..1025: mol_type = genomic DNA
agtcgagcggacagatgggagcttgctccctgatgttagcggcggacgggtgagtaacacgtgggtaacctgcctgtaagactgggataactccgggaaaccggggctaataccggatggttgtctgaaccgcatggttcagacataaaaggtggcttcggctaccacttacagatggacccgcggcgcattagctagttggtgaggtaacggctcaccaaggcgacgatgcgtagccgacctgagagggtgatcggccacactgggactgagacacggcccagactcctacgggaggcagcagtagggaatcttccgcaatggacgaaagtctgacggagcaacgccgcgtgagtgatgaaggttttcggatcgtaaagctctgttgttagggaagaacaagtgccgttcaaatagggcggcaccttgacggtacctaaccagaaagccacggctaactacgtgccagcagccgcggtaatacgtaggtggcaagcgttgtccggaattattgggcgtaaagggctcgcaggcggtttcttaagtctgatgtgaaagcccccggctcaaccggggagggtcattggaaactggggaacttgagtgcagaagaggagagtggaattccacgtgtagcggtgaaatgcgtagagatgtggaggaacaccagtggcgaaggcgactctctggtctgtaactgacgctgaggagcgaaagcgtggggagcgaacaggattagataccctggtagtccacgccgtaaacgatgagtgctaagtgttagggggtttccgccccttagtgctgcagctaacgcattaagcactccgcctggggagtacggtcgcaagactgaaactcaaaggaattgacgggggcccgcacaagcggtggagcatgtggtttaattcgaagcaacgcgaagaaccttaccaggtcttgacatcctctgacaatcctagagataggacgtccccttcgggggcagagtgacaggtggtgcatggttgtcgtcagctcgtgtc

SEQ ID NO: 3 - DNA, 1544 bp, Bacillus sp.
  source 1..1544: mol_type = genomic DNA
ttatcggagagtttgatcctggctcaggacgaacgctggcggcgtgcctaatacatgcaagtcgagcggacagatgggagcttgctccctgatgttagcggcggacgggtgagtaacacgtgggtaacctgcctgtaagactgggataactcgggaaaccgggctaatgatggttgtctgaaccgcatggttcagacataaaaggtggcttcggctaccacttacagatggacccgcggcgcattagctagttggtgaggtaacggctcaccaaggcgacgatgcgtagccgacctgagagggtgatcggccacactgggactgagacacggcccagactcctacgggaggcagcagtagggaatcttccgcaatggacgaaagtctgacggagcaacgccgcgtgagtgatgaaggttttcggatcgtaaagctctgttgttagggaagaacaagtgccgttcaaatagggcggcaccttgacggtacctaaccagaaagccacggctaactacgtgccagcagccgcggtaatacgtaggtggcaagcgttgtccggaattattgggcgtaaagggctcgcaggcggtttcttaagtctgatgtgaaagcccccggctcaaccggggagggtcattggaaactggggaacttgagtgcagaagaggagagtggaattccacgtgtagcggtgaaatgcgtagagatgtggaggaacaccagtggcgaaggcgactctctggtctgtaactgacgctgaggagcgaaagcgtggggagcgaacaggattagataccctggtagtccacgccgtaaacgatgagtgctaagtgttagggggtttccgccccttagtgctgcagctaacgcattaagcactccgcctggggagtacggtcgcaagactgaaactcaaaggaattgacgggggcccgcacaagcggtggagcatgtggtttaattcgaagcaacgcgaagaaccttaccaggtcttgacatcctctgacaatcctagagataggacgtccccttcgggggcagagtgacaggtggtgcatggttgtcgtcagctcgtgtcgtgagatgttgggttaagtcccgcaacgagcgcaacccttgatcttagttgccagcattcagttgggcactctaaggtgactgccggtgacaaaccggaggaaggtggggatgacgtcaaatcatcatgccccttatgacctgggctacacacgtgctacaatggacagaacaaagggcagcgaaaccgcgaggttaagccaatcccacaaatctgttctcagttcggatcgcagtctgcaactcgactgcgtgaagctggaatcgctagtaatcgcggatcagcatgccgcggtgaatacgttcccgggccttgtacacaccgcccgtcacaccacgagagtttgtaacacccgaagtcggtgaggtaacctttatggagccagccgccgaaggtgggacagatgattggggtgaagtcgtaacaaggtagccgtatcggaaggtgcggctggatcacctccttt

SEQ ID NO: 4 - DNA, 1015 bp, Bacillus sp.
  source 1..1015: mol_type = genomic DNA
agtcgagcggacagatgggagcttgctccctgatgttagcggcggacgggtgagtaacacgtgggtaacctgcctgtaagactgggataactccgggaaaccggggctaataccggatggttgtctgaaccgcatggttcagacataaaaggtggcttcggctaccacttacagatggacccgcggcgcattagctagttggtgaggtaacggctcaccaaggcgacgatgcgtagccgacctgagagggtgatcggccacactgggactgagacacggcccagactcctacgggaggcagcagtagggaatcttccgcaatggacgaaagtctgacggagcaacgccgcgtgagtgatgaaggttttcggatcgtaaagctctgttgttagggaagaacaagtgccgttcaaatagggcggcaccttgacggtacctaaccagaaagccacggctaactacgtgccagcagccgcggtaatacgtaggtggcaagcgttgtccggaattattgggcgtaaagggctcgcaggcggtttcttaagtctgatgtgaaagcccccggctcaaccggggagggtcattggaaactggggaacttgagtgcagaagaggagagtggaattccacgtgtagcggtgaaatgcgtagagatgtggaggaacaccagtggcgaaggcgactctctggtctgtaactgacgctgaggagcgaaagcgtggggagcgaacaggattagataccctggtagtccacgccgtaaacgatgagtgctaagtgttagggggtttccgccccttagtgctgcagctaacgcattaagcactccgcctggggagtacggtcgcaagactgaaactcaaaggaattgacgggggcccgcacaagcggtggagcatgtggtttaattcgaagcaacgcgaagaaccttaccaggtcttgacatcctctgacaatcctagagataggacgtccccttcgggggcagagtgacaggtggtgcatggttgtcgtc

SEQ ID NO: 5 - DNA, 989 bp, Bacillus sp.
  source 1..989: mol_type = genomic DNA
agtcgagcggacagatgggagcttgctccctgatgttagcggcggacgggtgagtaacacgtgggtaacctgcctgtaagactgggataactccgggaaaccggggctaataccggatggttgtctgaaccgcatggttcagacataaaaggtggcttcggctaccacttacagatggacccgcggcgcattagctagttggtgaggtaacggctcaccaaggcgacgatgcgtagccgacctgagagggtgatcggccacactgggactgagacacggcccagactcctacgggaggcagcagtagggaatcttccgcaatggacgaaagtctgacggagcaacgccgcgtgagtgatgaaggttttcggatcgtaaagctctgttgttagggaagaacaagtgccgttcaaatagggcggcaccttgacggtacctaaccagaaagccacggctaactacgtgccagcagccgcggtaatacgtaggtggcaagcgttgtccggaattattgggcgtaaagggctcgcaggcggtttcttaagtctgatgtgaaagcccccggctcaaccggggagggtcattggaaactggggaacttgagtgcagaagaggagagtggaattccacgtgtagcggtgaaatgcgtagagatgtggaggaacaccagtggcgaaggcgactctctggtctgtaactgacgctgaggagcgaaagcgtggggagcgaacaggattagataccctggtagtccacgccgtaaacgatgagtgctaagtgttagggggtttccgccccttagtgctgcagctaacgcattaagcactccgcctggggagtacggtcgcaagactgaaactcaaaggaattgacgggggcccgcacaagcggtggagcatgtggtttaattcgaagcaacgcgaagaaccttaccaggtcttgacatcctctgacaatcctagagataggacgtccccttcgggggcaga

SEQ ID NO: 6 - DNA, 1025 bp, Bacillus sp.; identical to SEQ ID NO: 2
  source 1..1025: mol_type = genomic DNA

SEQ ID NO: 7 - DNA, 1374 bp, Paenibacillus sp.
  source 1..1374: mol_type = genomic DNA
atccttttcctgcatgggagaaggaggaaagacggagcaatctgtcacttgtggatgggcctgcggcgcattagctagttggtggggtaaaggcctaccaaggcgacgatgcgtagccgacctgagagggtgatcggccacactgggactgagacacggcccagactcctacgggaggcagcagtagggaatcttccgcaatgggcgaaagcctgacggagcaacgccgcgtgagtgatgaaggttttcggatcgtaaagctctgttgccagggaagaacgtcttgtagagtaactgctacaagagtgacggtacctgagaagaaagccccggctaactacgtgccagcagccgcggtaatacgtagggggcaagcgttgtccggaattattgggcgtaaagcgcgcgcaggcggctctttaagtctggtgtttaatcccgaggctcaacttcgggtcgcactggaaactggggagcttgagtgcagaagaggagagtggaattccacgtgtagcggtgaaatgcgtagagatgtggaggaacaccagtggcgaaggcgactctctgggctgtaactgacgctgaggcgcgaaagcgtggggagcaaacaggattagataccctggtagtccacgccgtaaacgatgaatgctaggtgttaggggtttcgatacccttggtgccgaagttaacacattaagcattccgcctggggagtacggtcgcaagactgaaactcaaaggaattgacggggacccgcacaagcagtggagtatgtggtttaattcgaagcaacgcgaagaaccttaccaggtcttgacatccctctgaccggtctagagatagacctttccttcgggacagaggagacaggtggtgcatggttgtcgtcagctcgtgtcgtgagatgttgggttaagtcccgcaacgagcgcaacccttatgcttagttgccagcaggtcaagctgggcactctaagcagactgccggtgacaaaccggaggaaggtggggatgacgtcaaatcatcatgccccttatgacctgggctacacacgtactacaatggccggtacaacgggaagcgaaatcgcgaggtggagccaatcctagaaaagccggtctcagttcggattgtaggctgcaactcgcctacatgaagtcggaattgctagtaatcgcggatcagcatgccgcggtgaatacgttcccgggtcttgtacacaccgcccgtcacaccacgagagtttacaacacccgaagtcggtggggtaacccgcaagggagccagccgccgaaggtggggtagatgattggggtgaagtcgtaacaaggtagccgtatcggaaggtgcggctggatcacctcctttc

SEQ ID NO: 8 - DNA, 1547 bp, Paenibacillus sp.
  source 1..1547: mol_type = genomic DNA
gagtttgatcctggctcaggacgaacgctggcggcgtgcctaatacatgcaagtcgagcggggttatttagaagcttgcttctaaataacctagcggcggacgggtgagtaacacgtaggcaacctgcccacaagacagggataactaccggaaacggtagctaatacccgatacatccttttcctgcatgggagaaggaggaaagacggagcaatctgtcacttgtggatgggcctgcggcgcattagctagttggtggggtaaaggcctaccaaggcgacgatgcgtagccgacctgagagggtgatcggccacactgggactgagacacggcccagactcctacgggaggcagcagtagggaatcttccgcaatgggcgaaagcctgacggagcaacgccgcgtgagtgatgaaggttttcggatcgtaaagctctgttgccagggaagaacgtcttatagagtaactgctataagagtgacggtacctgagaagaaagccccggctaactacgtgccagcagccgcggtaatacgtagggggcaagcgttgtccggaattattgggcgtaaagcgcgcgcaggcggctctttaagtctggtgtttaatcccgaggctcaacttcgggtcgcactggaaactggggagcttgagtgcagaagaggagagtggaattccacgtgtagcggtgaaatgcgtagagatgtggaggaacaccagtggcgaaggcgactctctgggctgtaactgacgctgaggcgcgaaagcgtggggagcaaacaggattagataccctggtagtccacgccgtaaacgatgaatgctaggtgttaggggtttcgatacccttggtgccgaagttaacacattaagcattccgcctggggagtacggtcgcaagactgaaactcaaaggaattgacggggacccgcacaagcagtggagtatgtggtttaattcgaagcaacgcgaagaaccttaccaggtcttgacatccctctgaccgctgtagagatatggctttccttcgggacagaggagacaggtggtgcatggttgtcgtcagctcgtgtcgtgagatgttgggttaagtcccgcaacgagcgcaacccttatgcttagttgccagcaggtcaagctgggcactctaagcagactgccggtgacaaaccggaggaaggtggggatgacgtcaaatcatcatgccccttatgacctgggctacacacgtactacaatggccggtacaacgggaagcgaagccgcgaggtggagccaatcctagaaaagccggtctcagttcggattgcaggctgcaactcgcctgcatgaagtcggaattgctagtaatcgcggatcagcatgccgcggtgaatacgttcccgggtcttgtacacaccgcccgtcacaccacgagagtttacaacacccgaagtcggtgaggtaaccgcaaggggccagccgccgaaggtggggtagatgattggggtgaagtcgtaacaaggtagccgtatcggaaggtgcggctggatcacctcctttc

SEQ ID NO: 9 - DNA, 986 bp, Bacillus sp.
  source 1..986: mol_type = genomic DNA
agtcgagcggacagatgggagcttgctccctgatgttagcggcggacgggtgagtaacacgtgggtaacctgcctgtaagactgggataactccgggaaaccggggctaataccggatggttgtctgaaccgcatggttcagacataaaaggtggcttcggctaccacttacagatggacccgcggcgcattagctagttggtgaggtaacggctcaccaaggcgacgatgcgtagccgacctgagagggtgatcggccacactgggactgagacacggcccagactcctacgggaggcagcagtagggaatcttccgcaatggacgaaagtctgacggagcaacgccgcgtgagtgatgaaggttttcggatcgtaaagctctgttgttagggaagaacaagtgccgttcaaatagggcggcaccttgacggtacctaaccagaaagccacggctaactacgtgccagcagccgcggtaatacgtaggtggcaagcgttgtccggaattattgggcgtaaagggctcgcaggcggtttcttaagtctgatgtgaaagcccccggctcaaccggggagggtcattggaaactggggaacttgagtgcagaagaggagagtggaattccacgtgtagcggtgaaatgcgtagagatgtggaggaacaccagtggcgaaggcgactctctggtctgtaactgacgctgaggagcgaaagcgtggggagcgaacaggattagataccctggtagtccacgccgtaaacgatgagtgctaagtgttagggggtttccgccccttagtgctgcagctaacgcattaagcactccgcctggggagtacggtcgcaagactgaaactcaaaggaattgacgggggcccgcacaagcggtggagcatgtggtttaattcgaagcaacgcgaagaaccttaccaggtcttgacatcctctgacaatcctagagataggacgtccccttcgggggc

SEQ ID NO: 10 - DNA, 1549 bp, Paenibacillus sp.
  source 1..1549: mol_type = genomic DNA
gagtttgatcctggctcaggacgaacgctggcggcgtgcctaatacatgcaagtcgagcgggattgtttagaagcttgcttctaaacaatctagcggcggacgggtgagtaacacgtaggcaacctgcccacaagacagggataactaccggaaacggtagctaatacccgatacatccttttcctgcatgggagaaggaggaaagacggagcaatctgtcacttgtggatgggcctgcggcgcattagctagttggtggggtaaaggcctaccaaggcgacgatgcgtagccgacctgagagggtgatcggccacactgggactgagacacggcccagactcctacgggaggcagcagtagggaatcttccgcaatgggcgaaagcctgacggagcaacgccgcgtgagtgatgaaggttttcggatcgtaaagctctgttgccagggaagaacgtcttgtagagtaactgctacaagagtgacggtacctgagaagaaagccccggctaactacgtgccagcagccgcggtaatacgtagggggcaagcgttgtccggaattattgggcgtaaagcgcgcgcaggcggctctttaagtctggtgtttaatcccgaggctcaacttcgggtcgcactggaaactggggagcttgagtgcagaagaggagagtggaattccacgtgtagcggtgaaatgcgtagagatgtggaggaacaccagtggcgaaggcgactctctgggctgtaactgacgctgaggcgcgaaagcgtggggagcaaacaggattagataccctggtagtccacgccgtaaacgatgaatgctaggtgttaggggtttcgatacccttggtgccgaagttaacacattaagcattccgcctggggagtacggtcgcaagactgaaactcaaaggaattgacggggacccgcacaagcagtggagtatgtggtttaattcgaagcaacgcgaagaaccttaccaggtcttgacatccctctgaccggtctagagatagacctttccttcgggacagaggagacaggtggtgcatggttgtcgtcagctcgtgtcgtgagatgttgggttaagtcccgcaacgagcgcaacccttatgcttagttgccagcaggtcaagctgggcactctaagcagactgccggtgacaaaccggaggaaggtggggatgacgtcaaatcatcatgccccttatgacctgggctacacacgtactacaatggccggtacaacgggaagcgaaatcgcgaggtggagccaatcctagaaaagccggtctcagttcggattgtaggctgcaactcgcctacatgaagtcggaattgctagtaatcgcggatcagcatgccgcggtgaatacgttcccgggtcttgtacacaccgcccgtcacaccacgagagtttacaacacccgaagtcggtggggtaacccgcaagggagccagccgccgaaggtggggtagatgattggggtgaagtcgtaacaaggtagccgtatcggaaggtgcggctggatcacctcctttc

SEQ ID NO: 11 - DNA, 1005 bp, Bacillus sp.
  source 1..1005: mol_type = genomic DNA
agtcgagcggacagatgggagcttgctccctgatgttagcggcggacgggtgagtaacacgtgggtaacctgcctgtaagactgggataactccgggaaaccggggctaataccggatggttgtttgaaccgcatggttcagacataaaaggtggcttcggctaccacttacagatggacccgcggcgcattagctagttggtgaggtaacggctcaccaaggcgacgatgcgtagccgacctgagagggtgatcggccacactgggactgagacacggcccagactcctacgggaggcagcagtagggaatcttccgcaatggacgaaagtctgacggagcaacgccgcgtgagtgatgaaggttttcggatcgtaaagctctgttgttagggaagaacaagtgccgttcaaatagggcggcaccttgacggtacctaaccagaaagccacggctaactacgtgccagcagccgcggtaatacgtaggtggcaagcgttgtccggaattattgggcgtaaagggctcgcaggcggtttcttaagtctgatgtgaaagcccccggctcaaccggggagggtcattggaaactggggaacttgagtgcagaagaggagagtggaattccacgtgtagcggtgaaatgcgtagagatgtggaggaacaccagtggcgaaggcgactctctggtctgtaactgacgctgaggagcgaaagcgtggggagcgaacaggattagataccctggtagtccacgccgtaaacgatgagtgctaagtgttagggggtttccgccccttagtgctgcagctaacgcattaagcactccgcctggggagtacggtcgcaagactgaaactcaaaggaattgacgggggcccgcacaagcggtggagcatgtggtttaattcgaagcaacgcgaagaaccttaccaggtcttgacatcctctgacaatcctagagataggacgtccccttcgggggcagagtgacaggtggtgcat

SEQ ID NO: 12 - DNA, 1980 bp, Paenibacillus sp.
  source 1..1980: mol_type = genomic DNA
ctactctacgtattccgtgaaatctacgttttccacgatccagcgtttgcgcggatccaccttatcacccatcaaagtggacaccctacgttcagccttggctgcatcctctatctgaacgcgtaacaaggtgcgtgaatcgggattcatcgttgtttcccataactgatcagggttcatttccccaagtcctttatagcgctgaagctcaaaattccgtccaaattcttttaaataattatcaagctgctcgtcagtccaagcataacgcaccgtttcgagcttacccgactttcgagttattttatacaatggcggttgagcaataaatatgcgtcctgcatcaataagctctttcatgtaccgataaaagaacgtcaacaacagcacttgaatgtgcgcaccatctgtgtctgcatcggtcataatgatgattttggaataattgctgtcttccagcgaaaactctgttcctacccccgcaccaatagctgctgtaatagcacggtactcatcattcttcataatatccgccagtttggatttctccggattcatcggcttaccctttagcggtaagatggcctgaattttggaatcccgtccctgcttggctgatcctccagccgaatcgccttccacaataaacaactcattacgtgtaaaatccttggactgcgcaggcgacagtttaccattcaaattggaactttcactgcgctttttaccggaacgcatctcatcccgagctttacgtgcagcttcacgcgctctggatgcttgaactgccttcttgatcaaagtttgtgctatctgcggattttcttccaaaaaacgctgcatctgctcagatacgatggcatccactgtactccgtgccgaagcgctacccagttgatcctttgtctgaccgacaaattcaacctcagccatcttgacactgattacaaccatcatgccctcacgtagatcgttgccctccaagtttttatccttttctttcaacatcaccgttttccgggcatagtcgttcatgacacgagtgtaagcggttttgaatcccgtttcatgcgtacctccgccacgtgtcggaatggagttaacgaacgaagcaatcgtctctgtataacccgcattgtactggatggcaatctctacttcaatgtcttctttctcggcattaaagtgaataacgtcatgcagcacatccttgccctcattcagaaaagcaacaaactgacttgcgccaccctcataaaaatactcatctgactttccgctgcgttcgtctttaagttgaatacgaaggcccgaatttagaaaagcaatttcctgaaggcgctcagccaacgtatcgtagttaaaatgaatgcctgcttgaaaaacacgaatatccggtttaaatgtaattttcgagcccgtcttgttagtattgcccagcacttcaaggcctgtggtcggttccccgacatgctccacgcccttcttgtcctgccaatattcaaaccgctgacggtgaatcttgccgtcccggtaaatttctacttcaagccattccgaaagagcgttcgttacagatgcacctacaccgtgcagacccccggactttttatatcccgaaccgccaaacttgcctccggcgtgcaaaatggtgaatacaacctgaggcgtaggaatccccgttttgtgcattcctgtaggaataccgcgcccgttgtctgataccgtaatggaaccgtccttatgcattgtaatatcaatgcgagagcaaaacttggcgagatgttcatccaccgcgttgtctacaatttcccataccaaatgatgcagccccgaagaactggtgctcccgatgtacatgcccggccgtttgcgaactgccacaagcccttcgagcacttgaatgtcgtccgcgccatattctgaagctccgctttgtgtgccggacgctcccgcagacaagtcgattttgtcgaccat

SEQ ID NO: 13 - DNA, 350 bp, Bacillus sp.
  source 1..350: mol_type = genomic DNA
gaccggaacgattacgcacttcgttccggatccggaaatcttcaaagaaacaaccgtatacgactatgatctgctttcaaaccgtgtccgggaattggccttcctgacaaaaggcgtaaacatcacgattgaagacaaacgtgaaggacaagaacggaaaaacgagtaccactacgaaggcggaatcaaaagctatgttgagtacttaaaccgttccaaagaagtcgttcatgaagagccgatttatatcgaaggcgagaaagacggcataacggttgaagttgcattgcaatacaacgacagctatacaagcaatatttattctttcacgaataatatcaacacatacg

SEQ ID NO: 14 - DNA, 1917 bp, Bacillus sp.
  source 1..1917: mol_type = genomic DNA
atggaacagcagcaaaatagttatgatgagaatcagatacaggtattagaaggtttggaagctgttcgaaagagaccggggatgtacatcggatcaactaacagcaaaggccttcaccacttggtgtgggaaatcgtcgacaacagtattgacgaagccctggccggttattgtacagatattaacatcgagattgaaaaagataacagcattaccgttaaggacaacgggcgcggcattccggtcggtatccaggagaagatgggccgccctgcggttgaagtcatcatgaccgttctccacgccggcggtaaatttgacggaagcggatataaagtatccggcggtcttcacggtgtaggggcgtctgtcgtaaacgccttgtcgaccactcttgacgttacggttcatcgtgacggaaaaatccactatcaggcgtacgagcgcggtgtacctgtggccgatcttgaagtgatcggtgatactgataagaccggaacgattacgcacttcgttccggatccggaaattttcaaagaaacaaccgtatacgactatgatctgctttcaaaccgtgtccgggaattggccttcctgacaaaaggcgtaaacatcacgattgaagacaaacgtgaaggacaagaacggaaaaacgagtaccactacgaaggcggaatcaaaagctatgttgagtacttaaaccgttccaaagaagtcgttcatgaagagccgatttatatcgaaggcgagaaagacggcataacggttgaagttgcattgcaatacaacgacagctatacaagcaatatttattctttcacgaataatatcaacacatacgaaggcggcacgcacgaggccggatttaaaaccggtctgacccgtgtcataaacgactatgcaagaagaaaagggattttcaaagaaaatgatccgaatttaagcggggatgatgtgagagaagggctgactgccattatttcaattaagcaccctgatccgcaattcgaaggtcagacgaaaacgaagctcggcaactccgaagcgagaacgatcactgatacgctgttttcttctgcgctggaaacattccttcttgaaaatccggactcagcccgcaaaatcgttgaaaaaggtttaatggccgcaagagcgcggatggcagcgaaaaaagcgcgggaattgacccgccgcaaaagtgcgcttgagatttccaatctgccgggcaaactggcggactgttcttctaaagatccgagcatttccgagctgtatatcgtagagggtgactctgcgggcggatcagcgaaacagggacgggaccgtcatttccaagccattctgccgctgcgcggtaagattctgaacgttgagaaagccagacttgataagattctctcaaacaatgaggtcagatcaatgatcacggccctcggaacaggaatcggagaagattttaatcttgaaaaagcgcgttatcataaagtggtcatcatgacggatgccgatgttgacggcgcccacatcagaacgcttttattaacgttcttctacagatacatgcgggaaatcatcgaaaacggctatgtctacattgcccagccgccgctttataaagtgcagcagggaaaacgggtggaatacgcttataacgataagcagcttgatgagctgttaaaagagcttccgcaatcacctaagcccggcctccagcgttataaaggtcttggagaaatgaacgcgactcagctttgggaaacgacaatggaccctgcgaccagaacgcttctgcaagtcaatcttgaagatgcaatggacgctgacgagacttttgaaatgctgatgggtgacaaagtagaaccgcggagaaacttcatagaagcaaacgccagatacgtgaaaaatcttgatatttaa

SEQ ID NO: 15 - DNA, 255 bp, Bacillus sp.
  source 1..255: mol_type = genomic DNA
tcctgacaaaaggcgtaaacatcacgattgaagacaaacgtgaaggacaagaacggaaaaacgagtaccactacgaaggcggaatcaaaagctatgttgagtacttaaaccgttccaaagaagtcgttcatgaagagccgatttatatcgaaggcgagaaagacggcataacggttgaagttgcattgcaatacaacgacagctatacaagcaatatttattctttcacgaataatatcaacacatacgaaggcg

SEQ ID NO: 16 - DNA, 495 bp, Bacillus sp.
  source 1..495: mol_type = genomic DNA
cacggtgtaggggcatctgtcgtaaacgccttgtcgaccactcttgacgttacggttcatcgtgacggaaaaatccactatcaggcgtacgagcgcggtgtacctgtggccgatcttgaagtgatcggtgatactgataagaccggaacgattacgcacttcgttccggatccggaaatcttcaaagaaacaatcgtatacgactatgatctgctttcaaaccgtgtccgggaattggccttcctgacaaaaggcgtaaacatcacgattgaagacaaacgtgaaggacaagaacggaaaaacgagtaccactacgaaggcggaatcaaaagctatgttgagtacttaaaccgttccaaagaagtcgttcatgaagagccgatttatatcgaaggcgagaaagacggcataacggttgaagttgcattgcaatacaacgacagctatacaagcaatatttattctttcacgaataatatcaacacatacgaaggc

SEQ ID NO: 17 - DNA, 1980 bp, Paenibacillus sp.
  source 1..1980: mol_type = genomic DNA
ctactctacgtattccgtgaaatctacgttttccacgatccagcgcttgcgcggatccaccttatcacccatcaaagtggacaccctgcgttcagccttggctgcatcctctatctgaacgcgtaacaaggtgcgtgaatcgggattcatcgttgtttcccataactgatcagggttcatttccccaagtcctttatagcgctgaagctcaaaatttcgtccaaattcttttaaataattatcaagctgctcgtcagtccaagcataacgcaccgtttcgagcttacccgactttcgagttattttatacaatggcggttgagcaataaatatgcgtcctgcatcaataagctctttcatgtaccgataaaagaacgtcaacaacagcacttgaatgtgcgcaccatctgtatctgcatcggtcataatgatgattttggaataattgctgtcttccagcgaaaactctgttcctactcccgcaccaatagctgctgtaatagcacggtactcatcattcttcataatatccgccagtttggatttttccggattcatcggcttgccctttagcggcaatatggcctgaattttggaatcccgtccctgcttggctgaacctccagccgaatcgccttccacaataaacaactcattacgtgtaaaatccttggactgcgcaggcgacagtttaccattcaaattggaactttcactgcgctttttaccggaacgcatctcatctcgagctttacgtgcagcttcacgcgctctggatgcttgaactgccttcttgatcaaagtttgtgctatctgcggattttcttccaaaaaacgctgcatctgctcagatacgatggcatccactgtactccgtgccgaagcgctacccagctgatcctttgtctggccgacaaattcaacttcagccattttgacactgattacagccatcatgccctcacgtagatcgttgccctccaagtttttatccttttctttcaacatcaccgttttgcgcgcatagtcgttcatgacacgagtgtaagcggttttgaatcccgtttcatgcgtacctccgccacgtgtcggaatggagttaacgaacgaagcaatcgtctctgtataaccagcattgtactggatggcaatctctacttcaatgtcttctttctcggcattaaagtgaataacgtcatgtagcacatccttgccctcattcagaaaagcaacaaactgacttgcgccaccctcataaaaatactcatctgactttccgctgcgttcgtctttaagttgaatacgaaggcccgaatttagaaaagcaatttcctgaaggcgctcagccaacgtatcgtagttaaaatgaatgcctgcctgaaaaacacgaatatccggtttaaatgtaattttcgagcccgtcttgttagtattgcccagcacttcaaggcctgtggtcggttctccgacatgctccacgcccttcttgtcctgccaatattcaaaccgctgacggtgaatcttgccgtcccggtaaatttctacttcaagccattccgaaagagcgttcgttacagacgcacctacaccgtgcagacccccggactttttatatcccgaaccgccaaacttacctccggcgtgcaaaatggtgaatacaacctgaggcgtaggaattcccgttttgtgcattcctgtaggaataccgcgcccgttgtctgatactgtaacggaaccgtccttatgcattgtaatatcaatgcgagagcaaaacttggcgagatgttcatccaccgcgttgtctacaatttcccataccaaatgatgcagtcccgaagaactggtgctcccgatgtacatgcccggccgtttgcgaactgccacaagcccttcgagcacttgaatgtcgtccgcgccatattctgaagctccgctttgtgtgccggatactcccgcagacaagtcgattttgtcgaccat

SEQ ID NO: 18 - DNA, 1980 bp, Paenibacillus sp.
  source 1..1980: mol_type = genomic DNA
ctactctacgtattccgtgaaatccacgttttccacgatccagcgcttacgtggatctaccttgtcacccatcaatgtggacacacggcgttcagctttggcagcatcctcaatttgaacgcgcaacagggtgcgtgattcgggattcattgtcgtttcccataactgatcaggattcatctccccgagtcctttataacgttgaagctcaaaattccgtccaaattcttttaggtaattatcaagctgctcgtcagtccaggcataacgaaccgtttcgagcttacccgacttgcgggttattttatacaatggcggctgagcaataaatatgcgtcctgcatcaatgagttctttcatgtaccgataaaagaacgtcaacaacagtacttgaatgtgcgcgccgtccgtatctgcgtcggtcataatgatgattttggaataattgctgtcttccagcgagaactctgttcctacccccgcgccaatcgctgccgtaatagcacggtactcatcatttttcataatatcggcaagctttgacttttccggattcatcggcttgccctttaacggtaaaatagcctggatcttggaatctcgaccctgtttggccgatcctcccgccgaatcgccttccacgataaataattcattacgtgtaaaatctttagattgcgcaggcgacagcttaccattcaaattagaactttcactgcgcttcttgccagaacgcatttcgtcccgagccttacgcgcagcttcacgtgctttggacgcttgaactgcctttttaatcaaagtttgcgcaatctgtggattttcttccaagaaacgctgcatctgttcagatacgatggcatccactgtacttcgtgccgaagcactccccagctgatcttttgtctgaccgacaaattcaacctcagccatcttgacactgattacagccatcatgccctcacgtagatcgttaccctccaggtttttatccttttccttcaacagcgctgttttgcgtgcatagtcattcatcacacgagtgtaagcggttttgaagcctgtttcatgcgttcccccgccacgtgttggaatggagttaacgaacgaagcaatcgtctctgtgtaaccagcattgtattggatggcaatctctacttcaatgtcctctttctcagcattaaagtgaataacatcatgcagtacatccttgccctcattcaaaaaagcaacaaactgactcgctccaccctcataataatattcatctgactttccactgcgttcgtctttaagctgaatacgaaggccggaattcagaaaggcaatttcctgaaggcgctcagccagtgtatcatagttaaaatggatgcctgactgaaaaacgcgaatatccggtttaaatgtaacttttgagcccgtcttgttagtattgcccagcacttcaaggcctgtggtcggttcaccgacatgctccacgcccttcttgtcctgccaatattcgaaccgctgacggtgaatcttgccgtcccggtagatttccacttcaagccattccgaaagagcgttcgttacagacgcacctaccccatgcagacccccggactttttatatcccgaaccgccaaacttacctccggcgtgcaaaatggtgaatacaacttgaggcgtaggaattcccattttatgcattcccgtaggaataccgcgcccgttgtctgatactgtaatagagccgtccttatgcattgtgatatcaatgcgagagcaaaacttggcaagatgttcatccaccgcgttgtctacaatttcccataccaaatgatgcagtcccgaagaactggtgctcccgatgtacatgcccggccgtttgcgaactgccacaagcccttcgagcacttgaatgtcgtccgcgccatattctgaagctccgttctgtgtaccggaagctcccgcagacaagtcgattttgtcgaccat

SEQ ID NO: 19 - DNA, 312 bp, Bacillus sp.
  source 1..312: mol_type = genomic DNA
tcttcaaagaaacaatcgtatacgactatgatctgctttcaaaccgtgtccgggaattggccttcctgacaaaaggcgtaaacatcacgattgaagacaaacgtgaaggacaagaacggaaaaacgagtaccactacgaaggcggaatcaaaagctatgttgagtacttaaaccgttccaaagaagtcgttcatgaagagccgatttatatcgaaggcgagaaagacggcataacggttgaagttgcattgcaatacaacgacagctatacaagcaatatttattctttcacgaataatatcaacacatacg

SEQ ID NO: 20 - DNA, 1980 bp, Paenibacillus sp.; identical to SEQ ID NO: 17
  source 1..1980: mol_type = genomic DNA

SEQ ID NO: 21 - DNA, 321 bp, Bacillus sp.
  source 1..321: mol_type = genomic DNA
gaaatcttcaaagaaacaatcgtatacgactatgatctgctttcaaaccgtgtccgggaattggccttcctgacaaaaggcgtaaacatcacgattgaagacaaacgtgaaggacaagaacggaaaaacgagtaccactacgaaggcggaatcaaaagctatgttgagtacttaaaccgttccaaagaagtcgttcatgaagagccgatttatatcgaaggcgagaaagacggcataacggttgaagttgcgttgcaatacaacgacagctatacaagcaacatttattctttcacaaataacatcaacacatacgaaggc

SEQ ID NO: 22 - DNA, 3564 bp, Paenibacillus sp.
  source 1..3564: mol_type = genomic DNA
atgaggggtgagtttaagttggcaggacatcttgttcaatatggtcgacgcactcggcgcagttatgcacgtattaatgaggtactcgaggttccgaacctgattgagatccaacaaaaatcctatgattggtttttggaggaaggattacgggaaatgtttcgggatatttcaccaattcaagatttcactggaaatctgattttggagtttatcgactattctctcggagaacccaaatataccgttgacgacgcaaaggaacgcgacgttacgtatgcagcaccgcttcgggtaaaagtccggcttattaataaagagaccggggaagtgaaagagcaggaagtattcatgggagacttcccgctgatgactgaaacgggtacgtttattattaacggtgcggaacgggttattgtcagccagttggttcgctctcccagcgtctatttcagcacaaaagtcgacaagaatgcgaaaacaacatacaccgcaacggtaattcctaaccggggggcttggctcgaactggagatggatgcgaaggatattatctatgtccggattgaccgtacccgtaaaattccggttacggtgttgctgcgtgcacttggctttggcactgatgctgagattctggatttgctcggcaatgacgaatatatccgcaacacacttgataaagacaatacggattccacggagaaagcgctgattgaaatttatgagcgtcttcgcccgggtgagccacctacactggataacgcaaagagcttgcttgttgcacgcttctttgatccaaaacgttatgatctggccaacgtaggccgttacaaaatcaataaaaagcttcacatcaaaaaccgtctgttcaatcaacgtcttgctgagacattgattgatacaacaactggtgaaattatcgctgaagcaggacaaatggtggatcgtcgcctgttggacgagattctggcccaactggaggaatcagtaggacaccgcacgtatcatgttgctagcggcgtgctggaaagcaatgatattccacttcaaacgattgatgtgttctcgccaatcgaggacggtaaagtagtaaaactgattgctaacggaaatattgataaatcggttaagaatattacgcctgccgatattatttcctccatcagttattttattaacttgcttcacggtatcggaagtacggacgatattgaccatttgggtaaccgtcgtttacgttctgtaggtgagttgctccaaaaccagttccgtatcggtttatcccgtatggaacgcgtggtgcgtgaaagaatgtcgattcaggatgctaatgtaattacgccacaagcgttgattaacatacgtccagtaattgcttcgattaaagagttctttggtagctcgcagctgtcacagtttatggatcagacaaacccgcttgctgaattaacgcacaaacgtcgtctgtccgcactcggacccggcggtttgacgcgtgaacgcgcaggcatggaagtgcgtgacgtccatccaagtcactacggccgtatgtgtcctatcgagacaccagagggaccaaacattggtttgatcaactctttgtccacatttgcacgtatcaacgagtacggatttatcgaagctccttatcgttgggtagatccgaaaaccggaaaagttacagaccagattgattacctgactgctgatgaagaagataactacatcgtagctcaggcgaacgcggaattgacggaggaaaacacctttaaggatgaggtcgtcattgtccgttataacaaacagtctgataacattattccaatggctagtagccgtgttgattacatggacgtatcacctaaacaggtcgtatcagttgcgacagcactgattccgtttctggagaatgatgactctaaccgcgcattgatgggttccaatatgcaacgtcaggctgtcccactattgattccgaagtctccattggtcggaacaggaatggagcacaagtctgcaaaagattctggtgtttgcattgtatccaaatacaacggagttatcgaacgctcttcggctaacgaaatttggttgcgtcgtatcgaaactgtagatggtgctgaagtgaagggcgacattgttaagtataaattacacaaatttatgcgatctaaccaaggaacttgcattaaccaacgtccgattgtgaacagaggagatattgtcaaagttggcgatattcttgcagatggtccatctacggagatgggtgagttggcgttgggacgtaacgttgtcgttgccttcatgacttgggaaggttacaactacgaggatgcgatcctgctgagtgagaaactggtcaaggaggatgtatacacctcgatccatattgaggaatacgaatccgaggctcgtgacacgaaacttggacctgaagaaatcactcgtgacattccaaatgtcggtgaagaggcgcttcgcaacttggatgagcgtggaatcattcgtattggtgccgaaatcggtgcaggtgacattcttgttggtaaagttacacctaaaggtgtgactgaattgacagctgaggaacgtctcttacacgcaatctttggtgagaaggcacgcgaggttcgcgatacttctttgagagttcctcacggaacagatgggattgttgtagatgtaaaggtgtttacacgtgaaaatggtgatgaactgccaccaggtgtaaatcagttggttcgtgtatatattgctcaaaaacgtaaaatctccgaaggcgataaaatggctggacgtcacggtaacaagggtgtcgttgcccgtattttgcctgaagaagatatgccgttcctgccggatggcacaccagtacaggtcgttctgaacccgctgggggtaccttcacggatgaacatcggacaggtgcttgaagtccatctgggtatggctgcaatgcgtcttggtattcatgtggcaactccagtattcgatggtgccaaggagtatgacgtgttcgatacaatggaagaggcaggcatgcagcgtaatggtaagactgtgttgtatgacggacgtacgggtgatcgttttgaacgtgaagttactgtcggtgtcatgcacatgatcaaactggcgcacatggtcgatgataaaatccatgctcgttctacaggtccttactctctcgttacgcagcaaccattgggtggtaaagctcaattcggtggacagcgcttcggggagatggaagtatgggcattggaagcctacggcgcggcgtacacgcttcaggaaattttgactgtgaaatccgatgatgtggttggacgtgttaaaacttacgaatccattgtcaaaggtgaaaatgtacctgaaccgggtgttccagaatcatttaaggtcttgatcaaagagctgcaaagcttgggtatggacgtgaagattctgtctgaagacgaacaagagattgaaatgagagagcttgatgatgaggatgacacaagcggcgataagctgagtttgaatctggaaggctctgaggttggcgtagagtag

SEQ ID NO: 23 - DNA, 756 bp, Bacillus sp.
  source 1..756: mol_type = genomic DNA
gaaacgcctgagggcccgaacatcggtttgatcaactcattgtcatcatttgcgaaagtaaaccgctttggtttcattgagacgccataccgccgcgttgatcctgaaacaggaaaagtaacgcctagaatcgactacctgactgctgatgaagaggataactatgtcgtagcccaagcgaatgctaagctgagcgatgacggttctttcttggatgacagcatcgtagcgcgtttcagaggggaaaacaccgttgtagcccgcaaccgcgtggattacatggacgtatctcctaaacaggttgtatctgctgcgacagcatgtattccgttcttggaaaacgatgactcgaaccgcgccctcatgggagcgaacatgcagcgtcaggctgtgcctttgatgcagccggaagctccgatcgtcggaacgggtatggaatacgtatccggtaaagactccggtgcagccgttatttgtaaacaccctggtatcgtagaacgggtggaagcgaaaaacgtatgggtgcgccgctatgaagaaattgacggccaaaaagtaaaaggcaacctggataagtacagcttgctgaaatttgtccgctccaaccaaggtacgtgctacaaccagcgtccgatcgtcagtgtcggcgatgaagtagtcaaaggagaaatccttgctgacggaccttcaatggagcttggtgaacttgctctcggccgcaacgtaatggtcggcttcatgacatgggatggttac

SEQ ID NO: 24 - DNA, 3246 bp, Bacillus sp.
  source 1..3246: mol_type = genomic DNA
atgggtgatttccctattatgacagataccggtacttttatcatcaacggtgcagaacgtgttatcgtatctcagcttgttcggtctccaagtgtatatttcagtggtaaagtagacaagaacggtaaaaaaggttttaccgcgactgtcattccaaaccgtggcgcatggttagaatacgaaactgatgcgaaagatgttgtgtatgtccgcattgatcgcacacgtaagttgccggttacggttcttttgcgtgctctcggcttcggttccgaccaagagattctcgatctcattggtgagaacgaatatctccgcaatacactggataaggacaacactgaaaacagtgacaaagcgcttcttgaaatctatgagcgccttcgtcccggagagccgcctacagtagaaaacgcaaaaagcttgctggattcccgtttcttcgatccgaagcgatacgaccttgcgaatgtaggacgctataaaattaataaaaagcttcatatcaagaaccgcctgtttaaccagcgccttgcagaaacactggtggatccggaaaccggtgaaattctcgctgaaaaagggcagattcttgacagaagaacacttgataaagtactgccatacttagaaaatggaatcggcttcagaaaactttatcctaacggcggcgttgtcgaggatgaagtgatgcttcaatccattaaaatctatgctcctaccgatgcagaaggagagcagacgatcaatgtgatcggcaatgcttacatcgaagaggcgattaaaaacattacgcctgctgatattatttcttctatcagctacttcttcaacctcctgcacggagtgggtgacactgatgatatcgaccatctcggaaaccgccgtctgcgttctgtaggtgagctcctgcaaaaccaattccgtatcggtttaagccggatggaacgtgtcgttcgtgaaagaatgtctattcaagacacgaatacaattacgccgcagcagctgattaacatcagacctgttattgcgtctattaaagagttcttcggaagctcacagctttctcaattcatggatcagacgaacccgcttgctgaattgacgcacaaacgccgtctgtcagctctcggaccgggcggtttgacacgtgagcgcgcaggtatggaagtacgtgacgttcactactctcactatggccgtatgtgtccgattgaaacgcctgagggcccgaacatcggtttgatcaactcattgtcatcatttgcgaaagtaaaccgctttggtttcattgagacgccataccgccgcgttgatcctgaaacaggaaaagtaacgcctagaatcgactacctgactgctgatgaagaggataactatgtcgtagcccaagcgaatgctaagctgagcgatgacggttctttcttggatgacagcatcgtagcgcgtttcagaggggaaaacaccgttgtagcccgcaaccgagtggattacatggacgtatctcctaaacaggttgtatctgctgcgacagcatgtattccgttcttggaaaacgatgactcgaaccgcgccctcatgggagcgaacatgcagcgtcaggctgtgcctttgatgcagccggaagctccgatcgtcggaacgggtatggaatacgtatccggtaaagactccggtgcagccgttatttgtaaacaccctggtatcgttgaacgggtggaagcgaaaaacgtatgggtgcgccgctatgaagaaattgacggtcaaaaagtaaaaggcaacctggataagtacagcttgctgaaatttgtccgctccaaccaaggtacgtgctacaatcagcgtccgatcgtcagtgtcggcgacgaagtagtcaaaggagaaatccttgctgacggaccttcaatggagcttggtgaacttgctctcggccgcaacgtaatggtcggcttcatgacatgggatggttacaactatgaggatgccatcatcatgagtgaacgccttgtgaaagatgatgtatacacatctattcacattgaagaatatgaatcagaagcacgtgatacaaagcttgggccggaagagatcacccgcgatattccaaacgtaggggaagatgcgcttcgcaatcttgatgaccgcggaattatccgtatcggtgcggaagtcaacgacggagaccttctcgtaggtaaagtaacgcctaaaggtgtaactgagcttacggctgaagaacgccttcttcatgcgatctttggagaaaaagcgcgtgaagtccgtgatacttctctccgtgtgcctcacggcggcggcggaattatccacgacgtaaaagtcttcaaccgtgaagacggcgacgaacttcctccgggagtgaaccagcttgtacgcgtatatatcgttcagaaacgtaagatttctgaaggtgataaaatggccggacgtcacggaaacaaaggggttatctcgaagattcttcctgaagaagatatgccttaccttcctgacggcacgccgatcgatatcatgcttaacccgctgggtgtaccatcacgtatgaatatcggtcaggtattagaacttcacatgggtatggctgcccgctacctcggcattcacatcgcgtcacctgtatttgacggcgcgcgtgaagaagatgtgtgggaaacacttgaagaagcaggcatgtcaagagacgctaaaacagttctttatgacggccgtacgggagaaccgttcgacaaccgtgtatctgtcggaatcatgtacatgatcaaactggcgcacatggttgatgataaacttcatgcccgttctacaggtccttactcacttgttacgcagcagcctctcggcggtaaagcccaattcggcggacagcgtttcggtgagatggaggtttgggcgcttgaagcttacggcgcagcttacacgcttcaagaaatcctgactgtgaagtccgatgacgtggtcggacgtgtgaaaacatatgaagccatcgtcaaaggcgacaatgttccagagcctggtgttccggaatcattcaaagtattgatcaaagagcttcaaagcttaggtatggacgtaaaaatcctttcaggcgatgaagaagaaatagaaatgagagatctagaagacgaggaagatgcgaaacaagctgacggccttgcattatcaggtgatgaagcgccggaagaaacagcatctccagacgttgaacgtgacgcagtaacgaaagaatag

SEQ ID NO: 25 - DNA, 756 bp, Bacillus sp.
  source 1..756: mol_type = genomic DNA
gaaacgcctgagggcccgaacatcggtttgatcaactcattgtcatcatttgcgaaagtaaaccgctttggtttcattgagacgccataccgccgcgttgatcctgaaacaggaaaagtaacgcctagaatcgactacctgactgctgatgaagaggataactatgtcgtagcccaagcgaatgctaagctgagcgatgacggttctttcttggatgacagcatcgtagcgcgtttcagaggggaaaacaccgttgtagcccgcaaccgcgtggattacatggacgtatctcctaaacaggttgtatctgctgcgacagcatgtattccgttcttggaaaacgatgactcgaaccgcgccctcatgggagcgaacatgcagcgtcaggctgtgcctttgatgcagccggaagctccgatcgtcggaacgggtatggaatacgtatccggtaaagactccggtgcagccgttatttgtaaacaccctggtatcgtagaacgggtggaagcgaaaaacgtatgggtgcgccgctatgaagaaattgacggccaaaaagtaaaaggcaacctggataagtacagcttgctgaaattcgtccgctccaaccaaggtacgtgctacaaccagcgtccgatcgtcagtgtcggcgatgaagtagtaaaaggagaaatccttgctgacggaccttcaatggagcttggtgaacttgctctcggccgcaacgtaatggtcggcttcatgacatgggatggttac

SEQ ID NO: 26 - DNA, 756 bp, Bacillus sp.
  source 1..756: mol_type = genomic DNA
gaaacgcctgagggcccgaacatcggtttgatcaactcattgtcatcatttgcgaaagtaaaccgctttggtttcattgagacgccataccgccgcgttgatcctgaaacaggaaaagtaacgcctagaatcgactacctgactgctgatgaagaggataactatgtcgtagcccaagcgaatgctaagctgagcgatgacggttctttcttggatgacagcatcgtagcgcgtttcagaggggaaaacaccgttgtagcccgcaaccgcgtggattacatggacgtatctcctaaacaggttgtatctgctgcgacagcatgtattccgttcttggaaaacgatgactcgaaccgtgccctcatgggagcgaacatgcagcgtcaggctgtgcctttgatgcagccggaagctccgatcgtcggaacgggtatggaatacgtatccggtaaagactccggtgcagccgttatttgtaaacaccctggtatcgttgaacgggtggaagcgaaaaacgtatgggtgcgccgctatgaagaaattgacggccaaaaagtaaaaggcaacctggataagtacagcttgctgaaatttgtccgctccaaccaaggtacgtgctacaaccagcgtccgatcgtcagtgtcggcgatgaagtagtcaaaggagaaatccttgctgacggaccttcaatggagcttggtgaacttgctctcggccgcaacgtaatggtcggcttcatgacatgggatggttac

SEQ ID NO: 27 - DNA, 756 bp, Bacillus sp.
  source 1..756: mol_type = genomic DNA
gaaacgcctgagggcccgaacatcggtttgatcaactcattgtcatcatttgcgaaagtaaaccgctttggtttcattgagacgccataccgccgcgttgatcctgaaacaggaaaagtaacgcctagaatcgactacttgactgctgatgaagaggataactatgtcgtagcccaagcgaatgctaagctgagcgatgacggttctttcttggatgacagcatcgtagcgcgtttcagaggggaaaacaccgttgtagcccgcaaccgcgtggattacatggacgtttctcctaaacaggttgtttctgctgcgacagcatgtattccgttcttggaaaacgatgactcgaaccgcgccctcatgggagcgaacatgcagcgtcaggctgtgcctttgatgcagccggaagctccgatcgtcggaacgggtatggaatacgtatccggtaaagactccggtgcagccgttatttgtaaacaccctggtatcgttgaacgggtggaagcgaaaaacgtatgggtgcgccgctatgaagaaattgacggccaaaaagtaaaaggcaacctggataagtacagcttgctgaaatttgtccgctccaaccaaggtacgtgctacaaccagcgtccgatcgtcagtgtcggcgatgaagtagtcaaaggagaaatccttgctgacggaccttcaatggagcttggtgaacttgctctcggccgcaacgtaatggtcggcttcatgacatgggatggttac

SEQ ID NO: 28 - DNA, 3564 bp, Paenibacillus sp.
  source 1..3564: mol_type = genomic DNA
atgaggggtgagtttaagttggcaggacatcttgttcaatatggtcgacgcactcggcgcagttatgcacgtattaatgaggtactcgaggttccgaacctgattgagatccaacaaaaatcctatgattggtttttggaggaaggattaagggaaatgtttcgggatatttctccaattcaggatttcactggaaatctgattctggagtttatcgactattctctcggagaacccaaatataccgttgacgacgcaaaggaacgcgacgttacgtatgcagcaccgcttcgggtaaaagtccggcttattaataaagaaaccggggaagtgaaagagcaggaagtattcatgggagacttcccgctgatgactgaaacgggtacgtttattattaacggtgcggaacgggttattgtcagccagttggttcgctctcccagcgtctatttcagcacaaaagtcgacaagaatgcgaaaacaacatacaccgcaacggtaattcctaaccggggggcttggctcgaactggagatggatgcgaaggatattatctatgtccggattgaccgtacccgtaaaattccggttacggtgttgctgcgtgcgctgggctttggcactgatgctgagattctggatttgctcggcaatgacgaatatatccgcaacacacttgataaagacaacacggattccaccgagaaagcgctgattgaaatttatgagcgtcttcgtccaggtgagccgcctacactggataacgcaaagagcttgctagttgctcgcttctttgatcctaaacgttatgatctggccaacgtaggccgttacaaaatcaataaaaagcttcacatcaaaaaccgtttgttcaatcaacgacttgctgagactttgattgatacaacaactggtgaaatcatcgctgaagccggtcaaatggtagatcgccgcctgttggacgagattttggcccaactggaggaatcagtaggacatcgtacgtatcatgttgcgagtggtgtgctagaaagcaatgatattccacttcaaacaatcgatgtattctcaccaattgaggatggcaaagtagtaaaactgattgctaatggaaatattgataaatcggttaagaatattacgcctgccgatattatttcctccatcagttattttattaacttgcttcacggaatcggaagtacggacgatattgaccatttgggtaaccgtcgtttgcgttctgtaggtgagttgctccaaaaccagttccgtatcggtttatcccgtatggaacgcgtggtgcgtgaaagaatgtcaattcaggatgctaatgtaattacgccacaagcgctgattaacatacgtccagtaattgcttcgattaaagagttctttggtagctcgcagctgtctcagtttatggatcagacgaacccgcttgctgaattaacgcacaaacgtcgtctgtccgcactcggacccggcggtttgacgcgcgaacgcgcgggcatggaagtgcgtgacgtccatccgagtcactacggccgtatgtgtcctatcgagacaccagagggaccaaacattggtttgatcaactctttgtccacttttgcacgcattaacgagtatggatttatcgaagctccttatcgttgggtagatccaaaaaccggaaaagttacagaccagattgattacctgactgctgatgaagaagataactacattgtagctcaggcgaatgcggaattgacggaggaaaacacctttaaggatgaggttgtcattgtccgttataacaaacagtctgataacattattccgatggctagtagccgtgtcgattacatggacgtatcgcctaaacaggtcgtatcggtcgcgactgcactgattccgttcttggagaatgatgactctaaccgcgcattgatgggttccaacatgcagcgtcaggctgtcccgcttctgattccgaagtctccattggtcggaacaggaatggagcacaagtctgcaaaagattccggtgtttgcgttgtatccaaatacaacggagttatcgaacgttcttcggctaacgaaatttggttgcgtcgtatcgaaactgtagatggcgctgaagtgaagggcgacattgttaagtataaattacacaaatttatgcgatctaaccaaggaacttgcatcaaccaacgtccgattgtgaacagaggagatattgtcaaagttggcgatattcttgcggatggtccatctacagagatgggtgagttggcgttgggacgtaacgttgtcgttgccttcatgacttgggaaggttacaactacgaggatgcgatcttgctgagtgagaaactggttaaggaagatgtatacacctcaatccatattgaggaatacgaatccgaggctcgtgacacgaagcttggacctgaagaaatcactcgcgacattccaaatgtcggtgaagaagcgcttcgcaacttggatgagcgtggaatcatacgtattggtgctgaaattggcgcaggtgacattctcgttggtaaagtaacacctaaaggtgtgactgaattgacagctgaagaacgtctcttacacgcaatctttggtgagaaggcacgcgaggttcgcgatacttctttgagagttcctcacggaacagacgggattgttgtagatgtaaaggtatttacacgtgaaaatggcgatgaactgccaccaggtgtaaatcagttggttcgagtatatattgctcaaaaacgtaaaatctccgaaggcgataaaatggctggacgtcacggtaacaagggtgtcgttgcccgtattctgcctgaagaagatatgccgttcctgccggatggcacaccagtacaggtcgttctgaacccgctgggcgtaccttcacggatgaacatcggacaggtgcttgaagtccatctgggtatggctgcaatgcgtcttggtattcatgtggcaactccagtattcgatggtgccaaggaatatgacgtattcgatacaatggaagaggcaggcatgcagcgtaatggtaagactgtgttgtatgacggacgtacgggtgatcgttttgaacgtgaagttactgtcggtgtcatgcacatgatcaaactggcgcacatggtcgatgataaaatccatgctcgttctacaggtccttactctctcgttacgcaacaaccattgggtggtaaagctcaatttggtggacagcgcttcggggagatggaagtatgggcattggaagcctacggcgcagcgtacacgcttcaggaaattttgactgtgaaatctgatgatgtggttggacgtgttaaaacttacgaatccattgtcaaaggtgaaaatgtacctgaaccgggtgttccagaatcatttaaggtcttgatcaaggagctgcaaagcttgggtatggacgtgaagattctgtctgaagacgaacaagagatcgaaatgagagagcttgatgatgaggatgacacaaccggcgataagctgagtttgaatctggaaggctctgaggttggcgtagagtag

SEQ ID NO: 29 - DNA, 3564 bp, Paenibacillus sp.
  source 1..3564: mol_type = genomic DNA
atgaggggtgagtttaagttggcaggacatcttgttcaatatggtcgacgcactcggcgcagttatgcacgtattaatgaggtactcgaggttcccaacctgattgagatccaacaaaaatcatatgattggtttttggaggaaggattacgggaaatgtttcgggatatttctccaattcaagatttcacaggaaatctgattttggagtttatcgattactctctcggagaacccaaatataccgttgacgacgcaaaagaacgcgacgttacgtatgcggcaccgcttcgggtaaaagtccggcttattaataaggaaaccggggaagtaaaagagcaggaagtattcatgggagacttcccgctgatgactgaaacgggtacgtttattattaacggtgcggaacgggttattgtcagccagttggttcgctctcccagcgtctatttcagcacaaaagtcgacaagaatgcgaaaacaacatacaccgcaacggtaattcctaaccggggggcttggctcgaactggagatggatgcgaaggatattatctatgtccggattgaccgtacccgtaaaattccggttacggtgttgctgcgtgcacttggctttggcactgatgctgagattctggatttgctcggcaatgacgaatatatccgcaacacacttgataaagacaacacggattccacggagaaagcgctgattgaaatttatgagcgtcttcgtccgggtgagccacctacattggataatgcaaagagcttgcttgttgcacgcttctttgatccaaaacgttatgatctggccaacgtaggccgttacaaaatcaataaaaagcttcacatcaaaaaccgtctgttcaatcaacgcctagctgagacactgattgatacaacaactggtgaaattatcgctgaagcagggcaaatggtagaccgccgcttgttggacgagattttggcacaactagaagagtcggttggacaccgtacgtatcatgttgctagtggcgtattggaaagcaatgatattccgcttcaaacgatcgatgtattctcgccaatcgaagacggtaaagtagtaaaactgattgccaatggaaatatcgataaatcggttaagaacattacgcctgccgatattatttcctccatcagttattttattaacttgcttcacggaatcggaagtacggacgacattgaccatttgggtaaccgtcgtttgcgttctgtaggtgagttgctccaaaatcagttccgtattggtctgtcccgtatggaacgcgtggtacgcgaaagaatgtcaattcaggatgctaatgtaattacgccacaagcgctgattaacatacgtccggtcattgcgtcgattaaagagttctttggtagctctcagctgtctcagttcatggatcagacaaacccgcttgctgaactaacacacaaacgtcgtttgtctgcactcggacccggcggtttgacgcgcgaacgcgcgggcatggaagtacgtgacgtccatccgagtcactacggccgtatgtgtcctatcgagacaccagagggaccaaacattggtttgatcaactctttgtcaacttttgcacgtatcaacgaatacggatttatcgaagctccttatcgctgggtagatccgaagactggaaaagttacagatcagattgattacctgactgctgatgaagaagataactacatcgttgctcaggcaaatgcggaattgacggaagaaaacacctttaaggatgaagtcgttattgttcgctataacaagcagtctgataacattattccaatggcaagtagccgtgtcgattacatggacgtatcacctaaacaggttgtatcggtcgcaactgctctgatcccgttcctggagaatgatgactcgaaccgtgcattgatgggttccaacatgcagcggcaggctgtcccattgctgattccgaaagcgcctttggtaggaacagggatggaacataagtctgcaaaagattccggtgtgtgcgttgtgtccaagtacaacggggtgattgaacgttcttcggctaacgaaatttggctgcgtcgtattgaaacagtagatggcgctgaagtcaaaggcgatattgttaagtataaattacacaaatttatgcgttctaaccaaggaacatgcatcaaccagcgtccaatcgtaaacagaggcgatattgtcaaagttggcgatattcttgctgacggtccttccaccgagatgggtgagttggcactgggacgtaacgttgtcgtagcgttcatgacttgggaaggttacaactacgaggatgcgatcttgctgagcgagaagctggttaaagaggatgtatatacctcgatccatatcgaggaatacgaatctgaagcccgtgatacgaaacttggaccagaagaaatcactcgtgatattccgaatgtcggtgaagaagcgcttcgcaatctagatgagcgcggcatcattcgcatcggtgctgaaatcgccgcaggtgacattcttgttggtaaagtaacacctaagggtgtaactgagttgacagctgaagaacgtctcttgcatgcaatcttcggtgagaaggcgcgcgaggttcgtgatacttccttgagagttcctcacggaaccgacggaatcgtcgtagatgttaaagtatttacacgtgaaaatggcgatgagctgccaccgggtgtaaaccagttggtacgcgtctatattgctcaaaaacgtaaaatttccgaaggcgataaaatggccggacgtcacggtaacaagggtgtcgttgcccgtattctgcctgaagaagatatgccgttcttgccagatggcacgccagtacaagtcgtactgaatccgctgggcgtaccttcacggatgaacatcggacaggtgcttgaagtgcatttgggtatggctgcaatgcgtcttggtattcatgtggcaactccagtattcgatggtgccaaggagtatgacgtatttgatacgatggaagaagcgggtatgcaacgcaatggtaagacagtgttgtatgatgggcgtacaggtgatcgttttgaacgtgaagttacggtcggtgtcatgcacatgatcaaactggcgcacatggtcgacgataagatccatgctcgttctacaggcccttactctctcgttacgcagcaaccgttgggtggtaaagctcaattcggtggtcagcgcttcggggagatggaagtatgggcactggaagcctacggtgcggcgtatacgcttcaggaaattttgactgtgaaatccgatgacgtggttggacgtgttaaaacttacgaatccatcgtcaaaggtgaaaatgtcccagaaccgggtgttcctgaatcattcaaggtcttgatcaaagagctgcaaagcttgggtatggacgtgaagattctgtctgaagacgaacaagagatcgaaatgagagagcttgatgatgaggatgatacaactggcgataagctgagtttgaatctggaaggctctgaggttggcgtagagtag

SEQ ID NO: 30 - DNA, 756 bp, Bacillus sp.; identical to SEQ ID NO: 23
  source 1..756: mol_type = genomic DNA

SEQ ID NO: 31 - DNA, 3564 bp, Paenibacillus sp.; identical to SEQ ID NO: 28
  source 1..3564: mol_type = genomic DNA

SEQ ID NO: 32 - DNA, 756 bp, Bacillus sp.
  source 1..756: mol_type = genomic DNA
gaaacgcctgagggcccgaacatcggtttgatcaactcattgtcatcatttgcgaaagtaaaccgctttggtttcattgagacgccataccgccgcgttgatcctgaaacaggaaaagtaacgcctagaatcgactacctgactgctgatgaagaggataactatgtcgtagcccaagcgaatgctaagctgagcgatgacggttctttcttggatgacagcatcgtagcgcgtttcagaggggaaaacaccgttgtagcccgcaaccgcgtggattacatggacgtatctcctaaacaggttgtatctgctgcgacagcatgtattccgttcttggaaaacgatgactcgaaccgcgccctcatgggagcgaacatgcagcgtcaggctgtgcctttgatgcagccggaagctccgatcgtcggaacgggtatggaatacgtatccggtaaagactccggtgcagccgttatttgtaaacaccctggtatcgttgaacgggtggaagcgaaaaacgtatgggtgcgccgctatgaagaaattgacggccaaaaagtaaaaggcaacctggataagtacagcttgctgaaatttgtccgctccaaccaaggtacgtgctacaaccagcgtccgatcgtcagtgtcggcgatgaagtagtcaaaggagaaatccttgctgacggaccttcaatggagcttggtgaacttgctctcggccgcaacgtaatggtcggcttcatgacatgggatggttac